European Patent Application EP 4 389 915 A1, published June 26, 2024. Title: Differential diagnosing of bipolar versus unipolar disorder in patient during depression phases using A to I RNA editing ZNF267 gene. Applicant: ALCEDIAG. Application EP. The sequence listing filed with the application follows.

SEQUENCE LISTING (16 sequences)

SEQ ID NO: 1 - DNA, 20 bp, Homo sapiens
  source 1..20: mol_type = unassigned DNA
ggctgaggtggtcttggatg

SEQ ID NO: 2 - DNA, 20 bp, Homo sapiens
  source 1..20: mol_type = unassigned DNA
cctcgccttccactgtgatt

SEQ ID NO: 3 - DNA, 23 bp, Homo sapiens
  source 1..23: mol_type = unassigned DNA
atacgggcaagctcttaactatt

SEQ ID NO: 4 - DNA, 20 bp, Homo sapiens
  source 1..20: mol_type = unassigned DNA
aacctccacctcctgttttc

SEQ ID NO: 5 - DNA, 22 bp, Homo sapiens
  source 1..22: mol_type = unassigned DNA
tttaaaagcttctccagtcagc

SEQ ID NO: 6 - DNA, 20 bp, Homo sapiens
  source 1..20: mol_type = unassigned DNA
tcctgagtagctgggaccat

SEQ ID NO: 7 - DNA, 20 bp, Homo sapiens
  source 1..20: mol_type = unassigned DNA
cagcacattctgttgccttc

SEQ ID NO: 8 - DNA, 20 bp, Homo sapiens
  source 1..20: mol_type = unassigned DNA
gtgactttgcccctcatttg

SEQ ID NO: 9 - DNA, 21 bp, Homo sapiens
  source 1..21: mol_type = unassigned DNA
aagcccatcctcgaactacag

SEQ ID NO: 10 - DNA, 20 bp, Homo sapiens
  source 1..20: mol_type = unassigned DNA
ttgctctgtcacctggactg

SEQ ID NO: 11 - DNA, 20 bp, Homo sapiens
  source 1..20: mol_type = unassigned DNA
gaaccaggctaggtgcaatg

SEQ ID NO: 12 - DNA, 20 bp, Homo sapiens
  source 1..20: mol_type = unassigned DNA
ccatgccctggtaatttttg

SEQ ID NO: 13 - DNA, 20 bp, Homo sapiens
  source 1..20: mol_type = unassigned DNA
gggatgtaaacgctgaatgg

SEQ ID NO: 14 - DNA, 20 bp, Homo sapiens
  source 1..20: mol_type = unassigned DNA
atgtgccaccatgactgact

SEQ ID NO: 15 - DNA, 21 bp, Homo sapiens
  source 1..21: mol_type = unassigned DNA
aggcttcacaaactgtcttgt

SEQ ID NO: 16 - DNA, 18 bp, Homo sapiens
  source 1..18: mol_type = unassigned DNA
ctcactgcaacctccgcc